European Patent Application EP 4 810 603 A1, published September 23, 2026. Title: 改変型酵素. Applicant: Amano Enzyme Inc. Application JP. The sequence listing filed with the application follows.

SEQUENCE LISTING (24 sequences)

SEQ ID NO: 1 - protein, 259 aa, Ralstonia pickettii
MLQGKTALVTGSTSGIGLGIACSLAAQGANIIMNGFGDVEAPKAQIAAAGKNAIRIGYHGADMSKPAEIEAMFAYADAEFGGVDILVNNAGIQYVANVEDFPTERWDAIIAINLTSAFHTTRLAVPGMKRKNWGRIINVASVHGLVASAQKSAYVAAKHGIVGFTKSVALETAQTGITSNAICPGWVLTPLVQKQIDARAEKDGLSALEAKTDLLMEKQPSREFVTPDQLGALAVFLCSDAAEQVRGVAWNMDGGWVAQ

SEQ ID NO: 2 - protein, 259 aa, synthetic construct
MLQGKTALVTGSTSGIGLGIACSLAAQGANIIMNGFGDVEAPKAQIMHLGKNAIRIGYHGADMSKPAEIEAMFAYADAEFGGVDILVNNAGIQYVANVEDFPTERWDAIIAINLTSAFHTTRLAVPGMKRKNWGRIINVASVHGLVASAQKSAYVAAKHGIVGFTKSVALETAQTGITSNAICPGWVLTPLVQKQIDARAEKDGLSALEAKTDLLMEKQPSREFVTPDQLGALAVFLCSDAAEQVRGVAWNMDGGWVAQ

SEQ ID NO: 3 - protein, 259 aa, synthetic construct
MLQGKTALVTGSTSGIGLGIACSLAAQGANIIMNGFGDVEAPKAQIAAAGKNFLGIGYHGADMSKPAEIEAMFAYADAEFGGVDILVNNAGIQYVANVEDFPTERWDAIIAINLTSAFHTTRLAVPGMKRKNWGRIINVASVHGLVASAQKSAYVAAKHGIVGFTKSVALETAQTGITSNAICPGWVLTPLVQKQIDARAEKDGLSALEAKTDLLMEKQPSREFVTPDQLGALAVFLCSDAAEQVRGVAWNMDGGWVAQ

SEQ ID NO: 4 - protein, 259 aa, synthetic construct
MLQGKTALVTGSTSGIGLGIACSLAAQGANIIMNGFGDVEAPKAQIAAAGKNLLEIGYHGADMSKPAEIEAMFAYADAEFGGVDILVNNAGIQYVANVEDFPTERWDAIIAINLTSAFHTTRLAVPGMKRKNWGRIINVASVHGLVASAQKSAYVAAKHGIVGFTKSVALETAQTGITSNAICPGWVLTPLVQKQIDARAEKDGLSALEAKTDLLMEKQPSREFVTPDQLGALAVFLCSDAAEQVRGVAWNMDGGWVAQ

SEQ ID NO: 5 - protein, 259 aa, synthetic construct
MLQGKTALVTGSTSGIGLGIACSLAAQGANIIMNGFGDVEAPKAQIAAAGKNPAMIGYHGADMSKPAEIEAMFAYADAEFGGVDILVNNAGIQYVANVEDFPTERWDAIIAINLTSAFHTTRLAVPGMKRKNWGRIINVASVHGLVASAQKSAYVAAKHGIVGFTKSVALETAQTGITSNAICPGWVLTPLVQKQIDARAEKDGLSALEAKTDLLMEKQPSREFVTPDQLGALAVFLCSDAAEQVRGVAWNMDGGWVAQ

SEQ ID NO: 6 - protein, 259 aa, synthetic construct
MLQGKTALVTGSTSGIGLGIACSLAAQGANIIMNGFGDVEAPKAQIAAAGKNEFFIGYHGADMSKPAEIEAMFAYADAEFGGVDILVNNAGIQYVANVEDFPTERWDAIIAINLTSAFHTTRLAVPGMKRKNWGRIINVASVHGLVASAQKSAYVAAKHGIVGFTKSVALETAQTGITSNAICPGWVLTPLVQKQIDARAEKDGLSALEAKTDLLMEKQPSREFVTPDQLGALAVFLCSDAAEQVRGVAWNMDGGWVAQ

SEQ ID NO: 7 - protein, 259 aa, synthetic construct
MLQGKTALVTGSTSGIGLGIACSLAAQGANIIMNGFGDVEAPKAQIAAAGKNAIRIGYHGADLSKPAEIEAMFAYADAEFGGVDILVNNAGIQYVANVEDFPTERWDAIIAINLTSAFHTTRLAVPGMKRKNWGRIINVASVHGLVASAQKSAYVAAKHGIVGFTKSVALETAQTGITSNAICPGWVLTPLVQKQIDARAEKDGLSALEAKTDLLMEKQPSREFVTPDQLGALAVFLCSDAAEQVRGVAWNMDGGWVAQ

SEQ ID NO: 8 - protein, 259 aa, synthetic construct
MLQGKTALVTGSTSGIGLGIACSLAAQGANIIMNGFGDVEAPKAQIAAAGKNAIRIGYHGADMSKPAEIEAMFAYADAEFIGVDILVNNAGIQYVANVEDFPTERWDAIIAINLTSAFHTTRLAVPGMKRKNWGRIINVASVHGLVASAQKSAYVAAKHGIVGFTKSVALETAQTGITSNAICPGWVLTPLVQKQIDARAEKDGLSALEAKTDLLMEKQPSREFVTPDQLGALAVFLCSDAAEQVRGVAWNMDGGWVAQ

SEQ ID NO: 9 - protein, 259 aa, synthetic construct
MLQGKTALVTGSTSGIGLGIACSLAAQGANIIMNGFGDVEAPKAQIAAAGKNAIRIGYHGADMSKPAEIEAMFAYADAEFGGVDILVNNAGIQYVANVEDFPTERWDAIIAINLTSAFHTTRLAVPGMKRKNWGRIINVASVHGLVGSAQKSAYVAAKHGIVGFTKSVALETAQTGITSNAICPGWVLTPLVQKQIDARAEKDGLSALEAKTDLLMEKQPSREFVTPDQLGALAVFLCSDAAEQVRGVAWNMDGGWVAQ

SEQ ID NO: 10 - protein, 259 aa, synthetic construct
MLQGKTALVTGSTSGIGLGIACSLAAQGANIIMNGFGDVEAPKAQIAAAGKNAIRIGYHGADMSKPAEIEAMFAYADAEFGGVDILVNNAGIQYVANVEDFPTERWDAIIAINLTSAFHTTRLAVPGMKRKNWGRIINVASVHGLVASAQKSAYVAAKHGIVGFTKSVALETAQTGITSNAICPGWVLTPLVQKQIDARAEKDGLSALEVKTDLLMEKQPSREFVTPDQLGALAVFLCSDAAEQVRGVAWNMDGGWVAQ

SEQ ID NO: 11 - protein, 259 aa, synthetic construct
MLQGKTALVTGSTSGIGLGIACSLAAQGANIIMNGFGDVEAPKAQIAAAGKNAIRIGYHGADMSKPAEIEAMFAYAAFEFGGVDILVNNAGIQYVANVEDFPTERWDAIIAINLTSAFHTTRLAVPGMKRKNWGRIINVASVHGLVASAQKSAYVAAKHGIVGFTKSVALETAQTGITSNAICPGWVLTPLVQKQIDARAEKDGLSALEAKTDLLMEKQPSREFVTPDQLGALAVFLCSAFAEQVRGVAWNMDGGWVAQ

SEQ ID NO: 12 - protein, 259 aa, synthetic construct
MLQGKTALVTGSTSGIGLGIACSLAAQGANIIMNGFGDVEAPKAQIAAAGKNAIRIGYHGADMSKPAEIEAMFAYADAEFGGVDILVNNAGIQYVANVEDFPTERWDAIIAINLTSAFHTTRLAVPGMKRKNWGRIINVASVHGLVASAQKSAYVAAKHGIVGFTKSVALETAQTGITSNAICPGWVLTPLVQKQIDARAEKDGLSALEAKTDLLMEKQPSREFVTPDQLGALAVFLCSDAAEQVRGVAVPIDGGWVAQ

SEQ ID NO: 13 - DNA, 780 bp, Ralstonia pickettii
  source 1..780: mol_type = other DNA
atgctgcaaggaaaaaccgccctcgtcacgggctcgaccagcgggattggtctgggtattgcctgttcgctggccgcgcagggcgccaacatcatcatgaatggctttggcgatgtggaagcacccaaggcgcagatcgcggccgcgggcaaaaatgccatccgcatcggatatcacggcgccgacatgagcaagccagccgagatcgaagcgatgttcgcctatgccgacgcagagtttggcggcgtggacatcctcgtcaacaacgccggcatccagtatgtggccaatgtcgaggatttcccgaccgaacgctgggacgccatcatcgccatcaacctcacctcggctttccacacgacgcggcttgctgtgccgggcatgaagcgcaagaactggggccgcatcatcaacgtcgcatcggtgcatgggttggtggcatcggcgcagaaatcggcgtacgtggcggccaaacacggtatcgtcggcttcaccaaatcggtggcgctggagaccgcacagacgggcatcacgtccaacgcgatctgcccgggctgggtgctgacgccgctggtgcagaagcagatcgatgcgcgcgccgagaaggatggcctgtccgcgctcgaagccaagacagatctgctgatggaaaagcagccttcgcgtgagttcgtgacgcccgatcagcttggcgcgctggcggtgtttctgtgcagcgacgcggcggagcaggtgcgcggcgtggcgtggaacatggatggtggctgggtggcgcagtaa

SEQ ID NO: 14 - DNA, 780 bp, synthetic construct
  source 1..780: mol_type = other DNA
atgctgcaaggaaaaaccgccctcgtcacgggctcgaccagcgggattggtctgggtattgcctgttcgctggccgcgcagggcgccaacatcatcatgaatggctttggcgatgtggaagcacccaaggcgcagatcatgcatttgggcaaaaatgccatccgcatcggatatcacggcgccgacatgagcaagccagccgagatcgaagcgatgttcgcctatgccgacgcagagtttggcggcgtggacatcctcgtcaacaacgccggcatccagtatgtggccaatgtcgaggatttcccgaccgaacgctgggacgccatcatcgccatcaacctcacctcggctttccacacgacgcggcttgctgtgccgggcatgaagcgcaagaactggggccgcatcatcaacgtcgcatcggtgcatgggttggtggcatcggcgcagaaatcggcgtacgtggcggccaaacacggtatcgtcggcttcaccaaatcggtggcgctggagaccgcacagacgggcatcacgtccaacgcgatctgcccgggctgggtgctgacgccgctggtgcagaagcagatcgatgcgcgcgccgagaaggatggcctgtccgcgctcgaagccaagacagatctgctgatggaaaagcagccttcgcgtgagttcgtgacgcccgatcagcttggcgcgctggcggtgtttctgtgcagcgacgcggcggagcaggtgcgcggcgtggcgtggaacatggatggtggctgggtggcgcagtaa

SEQ ID NO: 15 - DNA, 780 bp, synthetic construct
  source 1..780: mol_type = other DNA
atgctgcaaggaaaaaccgccctcgtcacgggctcgaccagcgggattggtctgggtattgcctgttcgctggccgcgcagggcgccaacatcatcatgaatggctttggcgatgtggaagcacccaaggcgcagatcgcggccgcgggcaaaaattttttgggtatcggatatcacggcgccgacatgagcaagccagccgagatcgaagcgatgttcgcctatgccgacgcagagtttggcggcgtggacatcctcgtcaacaacgccggcatccagtatgtggccaatgtcgaggatttcccgaccgaacgctgggacgccatcatcgccatcaacctcacctcggctttccacacgacgcggcttgctgtgccgggcatgaagcgcaagaactggggccgcatcatcaacgtcgcatcggtgcatgggttggtggcatcggcgcagaaatcggcgtacgtggcggccaaacacggtatcgtcggcttcaccaaatcggtggcgctggagaccgcacagacgggcatcacgtccaacgcgatctgcccgggctgggtgctgacgccgctggtgcagaagcagatcgatgcgcgcgccgagaaggatggcctgtccgcgctcgaagccaagacagatctgctgatggaaaagcagccttcgcgtgagttcgtgacgcccgatcagcttggcgcgctggcggtgtttctgtgcagcgacgcggcggagcaggtgcgcggcgtggcgtggaacatggatggtggctgggtggcgcagtaa

SEQ ID NO: 16 - DNA, 780 bp, synthetic construct
  source 1..780: mol_type = other DNA
atgctgcaaggaaaaaccgccctcgtcacgggctcgaccagcgggattggtctgggtattgcctgttcgctggccgcgcagggcgccaacatcatcatgaatggctttggcgatgtggaagcacccaaggcgcagatcgcggccgcgggcaaaaatctgcttgagatcggatatcacggcgccgacatgagcaagccagccgagatcgaagcgatgttcgcctatgccgacgcagagtttggcggcgtggacatcctcgtcaacaacgccggcatccagtatgtggccaatgtcgaggatttcccgaccgaacgctgggacgccatcatcgccatcaacctcacctcggctttccacacgacgcggcttgctgtgccgggcatgaagcgcaagaactggggccgcatcatcaacgtcgcatcggtgcatgggttggtggcatcggcgcagaaatcggcgtacgtggcggccaaacacggtatcgtcggcttcaccaaatcggtggcgctggagaccgcacagacgggcatcacgtccaacgcgatctgcccgggctgggtgctgacgccgctggtgcagaagcagatcgatgcgcgcgccgagaaggatggcctgtccgcgctcgaagccaagacagatctgctgatggaaaagcagccttcgcgtgagttcgtgacgcccgatcagcttggcgcgctggcggtgtttctgtgcagcgacgcggcggagcaggtgcgcggcgtggcgtggaacatggatggtggctgggtggcgcagtaa

SEQ ID NO: 17 - DNA, 780 bp, synthetic construct
  source 1..780: mol_type = other DNA
atgctgcaaggaaaaaccgccctcgtcacgggctcgaccagcgggattggtctgggtattgcctgttcgctggccgcgcagggcgccaacatcatcatgaatggctttggcgatgtggaagcacccaaggcgcagatcgcggccgcgggcaaaaatcctgcgatgatcggatatcacggcgccgacatgagcaagccagccgagatcgaagcgatgttcgcctatgccgacgcagagtttggcggcgtggacatcctcgtcaacaacgccggcatccagtatgtggccaatgtcgaggatttcccgaccgaacgctgggacgccatcatcgccatcaacctcacctcggctttccacacgacgcggcttgctgtgccgggcatgaagcgcaagaactggggccgcatcatcaacgtcgcatcggtgcatgggttggtggcatcggcgcagaaatcggcgtacgtggcggccaaacacggtatcgtcggcttcaccaaatcggtggcgctggagaccgcacagacgggcatcacgtccaacgcgatctgcccgggctgggtgctgacgccgctggtgcagaagcagatcgatgcgcgcgccgagaaggatggcctgtccgcgctcgaagccaagacagatctgctgatggaaaagcagccttcgcgtgagttcgtgacgcccgatcagcttggcgcgctggcggtgtttctgtgcagcgacgcggcggagcaggtgcgcggcgtggcgtggaacatggatggtggctgggtggcgcagtaa

SEQ ID NO: 18 - DNA, 780 bp, synthetic construct
  source 1..780: mol_type = other DNA
atgctgcaaggaaaaaccgccctcgtcacgggctcgaccagcgggattggtctgggtattgcctgttcgctggccgcgcagggcgccaacatcatcatgaatggctttggcgatgtggaagcacccaaggcgcagatcgcggccgcgggcaaaaatgagttttttatcggatatcacggcgccgacatgagcaagccagccgagatcgaagcgatgttcgcctatgccgacgcagagtttggcggcgtggacatcctcgtcaacaacgccggcatccagtatgtggccaatgtcgaggatttcccgaccgaacgctgggacgccatcatcgccatcaacctcacctcggctttccacacgacgcggcttgctgtgccgggcatgaagcgcaagaactggggccgcatcatcaacgtcgcatcggtgcatgggttggtggcatcggcgcagaaatcggcgtacgtggcggccaaacacggtatcgtcggcttcaccaaatcggtggcgctggagaccgcacagacgggcatcacgtccaacgcgatctgcccgggctgggtgctgacgccgctggtgcagaagcagatcgatgcgcgcgccgagaaggatggcctgtccgcgctcgaagccaagacagatctgctgatggaaaagcagccttcgcgtgagttcgtgacgcccgatcagcttggcgcgctggcggtgtttctgtgcagcgacgcggcggagcaggtgcgcggcgtggcgtggaacatggatggtggctgggtggcgcagtaa

SEQ ID NO: 19 - DNA, 780 bp, synthetic construct
  source 1..780: mol_type = other DNA
atgctgcaaggaaaaaccgccctcgtcacgggctcgaccagcgggattggtctgggtattgcctgttcgctggccgcgcagggcgccaacatcatcatgaatggctttggcgatgtggaagcacccaaggcgcagatcgcggccgcgggcaaaaatgccatccgcatcggatatcacggcgccgacctgagcaagccagccgagatcgaagcgatgttcgcctatgccgacgcagagtttggcggcgtggacatcctcgtcaacaacgccggcatccagtatgtggccaatgtcgaggatttcccgaccgaacgctgggacgccatcatcgccatcaacctcacctcggctttccacacgacgcggcttgctgtgccgggcatgaagcgcaagaactggggccgcatcatcaacgtcgcatcggtgcatgggttggtggcatcggcgcagaaatcggcgtacgtggcggccaaacacggtatcgtcggcttcaccaaatcggtggcgctggagaccgcacagacgggcatcacgtccaacgcgatctgcccgggctgggtgctgacgccgctggtgcagaagcagatcgatgcgcgcgccgagaaggatggcctgtccgcgctcgaagccaagacagatctgctgatggaaaagcagccttcgcgtgagttcgtgacgcccgatcagcttggcgcgctggcggtgtttctgtgcagcgacgcggcggagcaggtgcgcggcgtggcgtggaacatggatggtggctgggtggcgcagtaa

SEQ ID NO: 20 - DNA, 780 bp, synthetic construct
  source 1..780: mol_type = other DNA
atgctgcaaggaaaaaccgccctcgtcacgggctcgaccagcgggattggtctgggtattgcctgttcgctggccgcgcagggcgccaacatcatcatgaatggctttggcgatgtggaagcacccaaggcgcagatcgcggccgcgggcaaaaatgccatccgcatcggatatcacggcgccgacatgagcaagccagccgagatcgaagcgatgttcgcctatgccgacgcagagtttatcggcgtggacatcctcgtcaacaacgccggcatccagtatgtggccaatgtcgaggatttcccgaccgaacgctgggacgccatcatcgccatcaacctcacctcggctttccacacgacgcggcttgctgtgccgggcatgaagcgcaagaactggggccgcatcatcaacgtcgcatcggtgcatgggttggtggcatcggcgcagaaatcggcgtacgtggcggccaaacacggtatcgtcggcttcaccaaatcggtggcgctggagaccgcacagacgggcatcacgtccaacgcgatctgcccgggctgggtgctgacgccgctggtgcagaagcagatcgatgcgcgcgccgagaaggatggcctgtccgcgctcgaagccaagacagatctgctgatggaaaagcagccttcgcgtgagttcgtgacgcccgatcagcttggcgcgctggcggtgtttctgtgcagcgacgcggcggagcaggtgcgcggcgtggcgtggaacatggatggtggctgggtggcgcagtaa

SEQ ID NO: 21 - DNA, 780 bp, synthetic construct
  source 1..780: mol_type = other DNA
atgctgcaaggaaaaaccgccctcgtcacgggctcgaccagcgggattggtctgggtattgcctgttcgctggccgcgcagggcgccaacatcatcatgaatggctttggcgatgtggaagcacccaaggcgcagatcgcggccgcgggcaaaaatgccatccgcatcggatatcacggcgccgacatgagcaagccagccgagatcgaagcgatgttcgcctatgccgacgcagagtttggcggcgtggacatcctcgtcaacaacgccggcatccagtatgtggccaatgtcgaggatttcccgaccgaacgctgggacgccatcatcgccatcaacctcacctcggctttccacacgacgcggcttgctgtgccgggcatgaagcgcaagaactggggccgcatcatcaacgtcgcatcggtgcatgggttggtgggctcggcgcagaaatcggcgtacgtggcggccaaacacggtatcgtcggcttcaccaaatcggtggcgctggagaccgcacagacgggcatcacgtccaacgcgatctgcccgggctgggtgctgacgccgctggtgcagaagcagatcgatgcgcgcgccgagaaggatggcctgtccgcgctcgaagccaagacagatctgctgatggaaaagcagccttcgcgtgagttcgtgacgcccgatcagcttggcgcgctggcggtgtttctgtgcagcgacgcggcggagcaggtgcgcggcgtggcgtggaacatggatggtggctgggtggcgcagtaa

SEQ ID NO: 22 - DNA, 780 bp, synthetic construct
  source 1..780: mol_type = other DNA
atgctgcaaggaaaaaccgccctcgtcacgggctcgaccagcgggattggtctgggtattgcctgttcgctggccgcgcagggcgccaacatcatcatgaatggctttggcgatgtggaagcacccaaggcgcagatcgcggccgcgggcaaaaatgccatccgcatcggatatcacggcgccgacatgagcaagccagccgagatcgaagcgatgttcgcctatgccgacgcagagtttggcggcgtggacatcctcgtcaacaacgccggcatccagtatgtggccaatgtcgaggatttcccgaccgaacgctgggacgccatcatcgccatcaacctcacctcggctttccacacgacgcggcttgctgtgccgggcatgaagcgcaagaactggggccgcatcatcaacgtcgcatcggtgcatgggttggtggcatcggcgcagaaatcggcgtacgtggcggccaaacacggtatcgtcggcttcaccaaatcggtggcgctggagaccgcacagacgggcatcacgtccaacgcgatctgcccgggctgggtgctgacgccgctggtgcagaagcagatcgatgcgcgcgccgagaaggatggcctgtccgcgctcgaagtcaagacagatctgctgatggaaaagcagccttcgcgtgagttcgtgacgcccgatcagcttggcgcgctggcggtgtttctgtgcagcgacgcggcggagcaggtgcgcggcgtggcgtggaacatggatggtggctgggtggcgcagtaa

SEQ ID NO: 23 - DNA, 780 bp, synthetic construct
  source 1..780: mol_type = other DNA
atgctgcaaggaaaaaccgccctcgtcacgggctcgaccagcgggattggtctgggtattgcctgttcgctggccgcgcagggcgccaacatcatcatgaatggctttggcgatgtggaagcacccaaggcgcagatcgcggccgcgggcaaaaatgccatccgcatcggatatcacggcgccgacatgagcaagccagccgagatcgaagcgatgttcgcctatgccgacgcagagtttggcggcgtggacatcctcgtcaacaacgccggcatccagtatgtggccaatgtcgaggatttcccgaccgaacgctgggacgccatcatcgccatcaacctcacctcggctttccacacgacgcggcttgctgtgccgggcatgaagcgcaagaactggggccgcatcatcaacgtcgcatcggtgcatgggttggtggcatcggcgcagaaatcggcgtacgtggcggccaaacacggtatcgtcggcttcaccaaatcggtggcgctggagaccgcacagacgggcatcacgtccaacgcgatctgcccgggctgggtgctgacgccgctggtgcagaagcagatcgatgcgcgcgccgagaaggatggcctgtccgcgctcgaagccaagacagatctgctgatggaaaagcagccttcgcgtgagttcgtgacgcccgatcagcttggcgcgctggcggtgtttctgtgcagcgcttttgcggagcaggtgcgcggcgtggcgtggaacatggatggtggctgggtggcgcagtaa

SEQ ID NO: 24 - DNA, 780 bp, synthetic construct
  source 1..780: mol_type = other DNA
atgctgcaaggaaaaaccgccctcgtcacgggctcgaccagcgggattggtctgggtattgcctgttcgctggccgcgcagggcgccaacatcatcatgaatggctttggcgatgtggaagcacccaaggcgcagatcgcggccgcgggcaaaaatgccatccgcatcggatatcacggcgccgacatgagcaagccagccgagatcgaagcgatgttcgcctatgccgacgcagagtttggcggcgtggacatcctcgtcaacaacgccggcatccagtatgtggccaatgtcgaggatttcccgaccgaacgctgggacgccatcatcgccatcaacctcacctcggctttccacacgacgcggcttgctgtgccgggcatgaagcgcaagaactggggccgcatcatcaacgtcgcatcggtgcatgggttggtggcatcggcgcagaaatcggcgtacgtggcggccaaacacggtatcgtcggcttcaccaaatcggtggcgctggagaccgcacagacgggcatcacgtccaacgcgatctgcccgggctgggtgctgacgccgctggtgcagaagcagatcgatgcgcgcgccgagaaggatggcctgtccgcgctcgaagccaagacagatctgctgatggaaaagcagccttcgcgtgagttcgtgacgcccgatcagcttggcgcgctggcggtgtttctgtgcagcgacgcggcggagcaggtgcgcggcgtggcggtccctatcgatggtggctgggtggcgcagtaa